European Patent Application EP 4 786 588 A1, published August 5, 2026. Title: non-natural 5' untranslated region and use thereof. Applicant: HANMI PHARM. CO., LTD. The sequence listing filed with the application follows.

SEQUENCE LISTING (36 sequences)

SEQ ID NO: 1 - RNA, 50 nt, synthetic construct
  source 1..50: mol_type = other RNA
agccgtcttccatcgttacagtcaccgttttcgcattctgtctagccacc

SEQ ID NO: 2 - RNA, 50 nt, synthetic construct
  source 1..50: mol_type = other RNA
agaatccagtcaacgcatatccacgtatacccgaacacatcacagccacc

SEQ ID NO: 3 - RNA, 50 nt, synthetic construct
  source 1..50: mol_type = other RNA
agccccccaacactgacttaatcgctttaagttcctccaaacgagccacc

SEQ ID NO: 4 - RNA, 50 nt, synthetic construct
  source 1..50: mol_type = other RNA
agagcagaacgcgtaaccacaccatcgcaacatcccacttgatagccacc

SEQ ID NO: 5 - RNA, 70 nt, synthetic construct
  source 1..70: mol_type = other RNA
agaccagacacctaacagactagacattttaccgaaatccgcattaaccattctaactcgtatagccacc

SEQ ID NO: 6 - RNA, 70 nt, synthetic construct
  source 1..70: mol_type = other RNA
agatcactaacaccatataacgctatcttcctccttctccgacattccagtactcattccacaagccacc

SEQ ID NO: 7 - RNA, 70 nt, synthetic construct
  source 1..70: mol_type = other RNA
agtacccactccagataaactgacaaccatacgcgaacaacgacgaatcgtatcacacgcagaagccacc

SEQ ID NO: 8 - RNA, 70 nt, synthetic construct
  source 1..70: mol_type = other RNA
agcgagataacttacaaggagagagaagacgaggagagataaattagagagaaaacgagtaagagccacc

SEQ ID NO: 9 - RNA, 70 nt, synthetic construct
  source 1..70: mol_type = other RNA
agtaaactaaccactccatcacgtatatattcctctttcacacctttccattctcgaactaaccgccacc

SEQ ID NO: 10 - protein, 393 aa, Homo sapiens [sequence omitted]

SEQ ID NO: 11 - DNA, 17 bp, synthetic construct
  source 1..17: mol_type = other DNA
taatacgactcactata

SEQ ID NO: 12 - DNA, 61 bp, Homo sapiens
  source 1..61: mol_type = genomic DNA
agtgctccccatccaactaaactgtccctctgtccgaactaaactgcactgtcccagcacc

SEQ ID NO: 13 - DNA, 1179 bp, Homo sapiens
  source 1..1179: mol_type = genomic DNA
atggaagaacctcagtccgatccgagcgtcgagcctcccctgtcacaggaaactttcagtgacctgtggaaactgctgcccgagaataatgtactttcgcctctgcctagccaagcaatggatgatctgatgctgtctccagatgacatcgaacagtggtttacagaggatccagggcccgatgaggcaccacgaatgccagaggcggccccacctgttgcacccgcacctgcggctccaacacccgcagcccccgcccccgctccaagctggcctctcagtagttccgtgccatcacagaagacctatcaaggcagctacggatttcgcctcggatttctccattcaggcactgccaagtccgtgacttgtacgtacagccccgctctgaacaaaatgttctgtcagttggcgaagacatgtcctgtccagctttgggtagattctacccccccgccggggacacgggtgcgagccatggccatttataaacagtctcagcacatgaccgaggtcgtgcgcaggtgtcctcaccatgaacgatgctccgactccgacggcctggcccccccacagcacctgattcgcgtggaaggcaatcttcgtgtggagtacctcgatgatcggaacaccttcagacatagcgtggttgtgccttatgagccacccgaagttggaagcgactgtaccaccatccattacaactatatgtgcaacagtagctgcatgggtggcatgaatcggcggcctatcttgacaataatcactttagaggactcttccggaaacctgcttggcagaaattcattcgaggtccgtgtctgcgcctgcccgggcagggaccgcagaaccgaagaggagaatttacggaaaaagggggaaccccaccacgaactgccaccgggcagtaccaaaagggctctccctaataacacatcttcatcgccccagccaaagaagaaacccctcgacggagagtactttactctacaaattagggggagagaaagatttgagatgttccgcgaattgaacgaggccctggagttgaaagacgctcaagccggaaaggaaccaggtgggtctagggcccactcaagccatctgaagagtaagaaaggccagtccacttccaggcacaaaaagttaatgttcaagacggagggtcctgactctgac

SEQ ID NO: 14 - DNA, 158 bp, Homo sapiens
  source 1..158: mol_type = genomic DNA
gtgtgtggaggacaccctgaaccccccgctttcaaacaagttttcaaattgtttgaggtcaggatttctcaaactgattcctttctttgcatatgagtatttgaaaataaatattttcccagaatataaataaatcatcacatgattattttaactat

SEQ ID NO: 15 - DNA, 100 bp, synthetic construct
  source 1..100: mol_type = other DNA
aaaaaaaaaaaaaaaaaaaaaaaaaaaaaaaaaaaaaaaaaaaaaaaaaaaaaaaaaaaaaaaaaaaaaaaaaaaaaaaaaaaaaaaaaaaaaaaaaaaa

SEQ ID NO: 16 - RNA, 61 nt, synthetic construct
  source 1..61: mol_type = other RNA
agtcctccccatcctctccctctgtccctctgtccctctgaccctgcactgtcccagcacc

SEQ ID NO: 17 - RNA, 1398 nt, synthetic construct
  source 1..1398: mol_type = other RNA
agtcctccccatcctctccctctgtccctctgtccctctgaccctgcactgtcccagcaccatggaagaacctcagtccgatccgagcgtcgagcctcccctgtcacaggaaactttcagtgacctgtggaaactgctgcccgagaataatgtactttcgcctctgcctagccaagcaatggatgatctgatgctgtctccagatgacatcgaacagtggtttacagaggatccagggcccgatgaggcaccacgaatgccagaggcggccccacctgttgcacccgcacctgcggctccaacacccgcagcccccgcccccgctccaagctggcctctcagtagttccgtgccatcacagaagacctatcaaggcagctacggatttcgcctcggatttctccattcaggcactgccaagtccgtgacttgtacgtacagccccgctctgaacaaaatgttctgtcagttggcgaagacatgtcctgtccagctttgggtagattctacccccccgccggggacacgggtgcgagccatggccatttataaacagtctcagcacatgaccgaggtcgtgcgcaggtgtcctcaccatgaacgatgctccgactccgacggcctggcccccccacagcacctgattcgcgtggaaggcaatcttcgtgtggagtacctcgatgatcggaacaccttcagacatagcgtggttgtgccttatgagccacccgaagttggaagcgactgtaccaccatccattacaactatatgtgcaacagtagctgcatgggtggcatgaatcggcggcctatcttgacaataatcactttagaggactcttccggaaacctgcttggcagaaattcattcgaggtccgtgtctgcgcctgcccgggcagggaccgcagaaccgaagaggagaatttacggaaaaagggggaaccccaccacgaactgccaccgggcagtaccaaaagggctctccctaataacacatcttcatcgccccagccaaagaagaaacccctcgacggagagtactttactctacaaattagggggagagaaagatttgagatgttccgcgaattgaacgaggccctggagttgaaagacgctcaagccggaaaggaaccaggtgggtctagggcccactcaagccatctgaagagtaagaaaggccagtccacttccaggcacaaaaagttaatgttcaagacggagggtcctgactctgacgtgtgtggaggacaccctgaaccccccgctttcaaacaagttttcaaattgtttgaggtcaggatttctcaaactgattcctttctttgcatatgagtatttgaaaataaatattttcccagaatataaataaatcatcacatgattattttaactat

SEQ ID NO: 18 - RNA, 1387 nt, synthetic construct
  source 1..1387: mol_type = other RNA
agccgtcttccatcgttacagtcaccgttttcgcattctgtctagccaccatggaagaacctcagtccgatccgagcgtcgagcctcccctgtcacaggaaactttcagtgacctgtggaaactgctgcccgagaataatgtactttcgcctctgcctagccaagcaatggatgatctgatgctgtctccagatgacatcgaacagtggtttacagaggatccagggcccgatgaggcaccacgaatgccagaggcggccccacctgttgcacccgcacctgcggctccaacacccgcagcccccgcccccgctccaagctggcctctcagtagttccgtgccatcacagaagacctatcaaggcagctacggatttcgcctcggatttctccattcaggcactgccaagtccgtgacttgtacgtacagccccgctctgaacaaaatgttctgtcagttggcgaagacatgtcctgtccagctttgggtagattctacccccccgccggggacacgggtgcgagccatggccatttataaacagtctcagcacatgaccgaggtcgtgcgcaggtgtcctcaccatgaacgatgctccgactccgacggcctggcccccccacagcacctgattcgcgtggaaggcaatcttcgtgtggagtacctcgatgatcggaacaccttcagacatagcgtggttgtgccttatgagccacccgaagttggaagcgactgtaccaccatccattacaactatatgtgcaacagtagctgcatgggtggcatgaatcggcggcctatcttgacaataatcactttagaggactcttccggaaacctgcttggcagaaattcattcgaggtccgtgtctgcgcctgcccgggcagggaccgcagaaccgaagaggagaatttacggaaaaagggggaaccccaccacgaactgccaccgggcagtaccaaaagggctctccctaataacacatcttcatcgccccagccaaagaagaaacccctcgacggagagtactttactctacaaattagggggagagaaagatttgagatgttccgcgaattgaacgaggccctggagttgaaagacgctcaagccggaaaggaaccaggtgggtctagggcccactcaagccatctgaagagtaagaaaggccagtccacttccaggcacaaaaagttaatgttcaagacggagggtcctgactctgacgtgtgtggaggacaccctgaaccccccgctttcaaacaagttttcaaattgtttgaggtcaggatttctcaaactgattcctttctttgcatatgagtatttgaaaataaatattttcccagaatataaataaatcatcacatgattattttaactat

SEQ ID NO: 19 - RNA, 1387 nt, synthetic construct
  source 1..1387: mol_type = other RNA
agaatccagtcaacgcatatccacgtatacccgaacacatcacagccaccatggaagaacctcagtccgatccgagcgtcgagcctcccctgtcacaggaaactttcagtgacctgtggaaactgctgcccgagaataatgtactttcgcctctgcctagccaagcaatggatgatctgatgctgtctccagatgacatcgaacagtggtttacagaggatccagggcccgatgaggcaccacgaatgccagaggcggccccacctgttgcacccgcacctgcggctccaacacccgcagcccccgcccccgctccaagctggcctctcagtagttccgtgccatcacagaagacctatcaaggcagctacggatttcgcctcggatttctccattcaggcactgccaagtccgtgacttgtacgtacagccccgctctgaacaaaatgttctgtcagttggcgaagacatgtcctgtccagctttgggtagattctacccccccgccggggacacgggtgcgagccatggccatttataaacagtctcagcacatgaccgaggtcgtgcgcaggtgtcctcaccatgaacgatgctccgactccgacggcctggcccccccacagcacctgattcgcgtggaaggcaatcttcgtgtggagtacctcgatgatcggaacaccttcagacatagcgtggttgtgccttatgagccacccgaagttggaagcgactgtaccaccatccattacaactatatgtgcaacagtagctgcatgggtggcatgaatcggcggcctatcttgacaataatcactttagaggactcttccggaaacctgcttggcagaaattcattcgaggtccgtgtctgcgcctgcccgggcagggaccgcagaaccgaagaggagaatttacggaaaaagggggaaccccaccacgaactgccaccgggcagtaccaaaagggctctccctaataacacatcttcatcgccccagccaaagaagaaacccctcgacggagagtactttactctacaaattagggggagagaaagatttgagatgttccgcgaattgaacgaggccctggagttgaaagacgctcaagccggaaaggaaccaggtgggtctagggcccactcaagccatctgaagagtaagaaaggccagtccacttccaggcacaaaaagttaatgttcaagacggagggtcctgactctgacgtgtgtggaggacaccctgaaccccccgctttcaaacaagttttcaaattgtttgaggtcaggatttctcaaactgattcctttctttgcatatgagtatttgaaaataaatattttcccagaatataaataaatcatcacatgattattttaactat

SEQ ID NO: 20 - RNA, 1387 nt, synthetic construct
  source 1..1387: mol_type = other RNA
agccccccaacactgacttaatcgctttaagttcctccaaacgagccaccatggaagaacctcagtccgatccgagcgtcgagcctcccctgtcacaggaaactttcagtgacctgtggaaactgctgcccgagaataatgtactttcgcctctgcctagccaagcaatggatgatctgatgctgtctccagatgacatcgaacagtggtttacagaggatccagggcccgatgaggcaccacgaatgccagaggcggccccacctgttgcacccgcacctgcggctccaacacccgcagcccccgcccccgctccaagctggcctctcagtagttccgtgccatcacagaagacctatcaaggcagctacggatttcgcctcggatttctccattcaggcactgccaagtccgtgacttgtacgtacagccccgctctgaacaaaatgttctgtcagttggcgaagacatgtcctgtccagctttgggtagattctacccccccgccggggacacgggtgcgagccatggccatttataaacagtctcagcacatgaccgaggtcgtgcgcaggtgtcctcaccatgaacgatgctccgactccgacggcctggcccccccacagcacctgattcgcgtggaaggcaatcttcgtgtggagtacctcgatgatcggaacaccttcagacatagcgtggttgtgccttatgagccacccgaagttggaagcgactgtaccaccatccattacaactatatgtgcaacagtagctgcatgggtggcatgaatcggcggcctatcttgacaataatcactttagaggactcttccggaaacctgcttggcagaaattcattcgaggtccgtgtctgcgcctgcccgggcagggaccgcagaaccgaagaggagaatttacggaaaaagggggaaccccaccacgaactgccaccgggcagtaccaaaagggctctccctaataacacatcttcatcgccccagccaaagaagaaacccctcgacggagagtactttactctacaaattagggggagagaaagatttgagatgttccgcgaattgaacgaggccctggagttgaaagacgctcaagccggaaaggaaccaggtgggtctagggcccactcaagccatctgaagagtaagaaaggccagtccacttccaggcacaaaaagttaatgttcaagacggagggtcctgactctgacgtgtgtggaggacaccctgaaccccccgctttcaaacaagttttcaaattgtttgaggtcaggatttctcaaactgattcctttctttgcatatgagtatttgaaaataaatattttcccagaatataaataaatcatcacatgattattttaactat

SEQ ID NO: 21 - RNA, 1387 nt, synthetic construct
  source 1..1387: mol_type = other RNA
agagcagaacgcgtaaccacaccatcgcaacatcccacttgatagccaccatggaagaacctcagtccgatccgagcgtcgagcctcccctgtcacaggaaactttcagtgacctgtggaaactgctgcccgagaataatgtactttcgcctctgcctagccaagcaatggatgatctgatgctgtctccagatgacatcgaacagtggtttacagaggatccagggcccgatgaggcaccacgaatgccagaggcggccccacctgttgcacccgcacctgcggctccaacacccgcagcccccgcccccgctccaagctggcctctcagtagttccgtgccatcacagaagacctatcaaggcagctacggatttcgcctcggatttctccattcaggcactgccaagtccgtgacttgtacgtacagccccgctctgaacaaaatgttctgtcagttggcgaagacatgtcctgtccagctttgggtagattctacccccccgccggggacacgggtgcgagccatggccatttataaacagtctcagcacatgaccgaggtcgtgcgcaggtgtcctcaccatgaacgatgctccgactccgacggcctggcccccccacagcacctgattcgcgtggaaggcaatcttcgtgtggagtacctcgatgatcggaacaccttcagacatagcgtggttgtgccttatgagccacccgaagttggaagcgactgtaccaccatccattacaactatatgtgcaacagtagctgcatgggtggcatgaatcggcggcctatcttgacaataatcactttagaggactcttccggaaacctgcttggcagaaattcattcgaggtccgtgtctgcgcctgcccgggcagggaccgcagaaccgaagaggagaatttacggaaaaagggggaaccccaccacgaactgccaccgggcagtaccaaaagggctctccctaataacacatcttcatcgccccagccaaagaagaaacccctcgacggagagtactttactctacaaattagggggagagaaagatttgagatgttccgcgaattgaacgaggccctggagttgaaagacgctcaagccggaaaggaaccaggtgggtctagggcccactcaagccatctgaagagtaagaaaggccagtccacttccaggcacaaaaagttaatgttcaagacggagggtcctgactctgacgtgtgtggaggacaccctgaaccccccgctttcaaacaagttttcaaattgtttgaggtcaggatttctcaaactgattcctttctttgcatatgagtatttgaaaataaatattttcccagaatataaataaatcatcacatgattattttaactat

SEQ ID NO: 22 - RNA, 1407 nt, synthetic construct
  source 1..1407: mol_type = other RNA
agaccagacacctaacagactagacattttaccgaaatccgcattaaccattctaactcgtatagccaccatggaagaacctcagtccgatccgagcgtcgagcctcccctgtcacaggaaactttcagtgacctgtggaaactgctgcccgagaataatgtactttcgcctctgcctagccaagcaatggatgatctgatgctgtctccagatgacatcgaacagtggtttacagaggatccagggcccgatgaggcaccacgaatgccagaggcggccccacctgttgcacccgcacctgcggctccaacacccgcagcccccgcccccgctccaagctggcctctcagtagttccgtgccatcacagaagacctatcaaggcagctacggatttcgcctcggatttctccattcaggcactgccaagtccgtgacttgtacgtacagccccgctctgaacaaaatgttctgtcagttggcgaagacatgtcctgtccagctttgggtagattctacccccccgccggggacacgggtgcgagccatggccatttataaacagtctcagcacatgaccgaggtcgtgcgcaggtgtcctcaccatgaacgatgctccgactccgacggcctggcccccccacagcacctgattcgcgtggaaggcaatcttcgtgtggagtacctcgatgatcggaacaccttcagacatagcgtggttgtgccttatgagccacccgaagttggaagcgactgtaccaccatccattacaactatatgtgcaacagtagctgcatgggtggcatgaatcggcggcctatcttgacaataatcactttagaggactcttccggaaacctgcttggcagaaattcattcgaggtccgtgtctgcgcctgcccgggcagggaccgcagaaccgaagaggagaatttacggaaaaagggggaaccccaccacgaactgccaccgggcagtaccaaaagggctctccctaataacacatcttcatcgccccagccaaagaagaaacccctcgacggagagtactttactctacaaattagggggagagaaagatttgagatgttccgcgaattgaacgaggccctggagttgaaagacgctcaagccggaaaggaaccaggtgggtctagggcccactcaagccatctgaagagtaagaaaggccagtccacttccaggcacaaaaagttaatgttcaagacggagggtcctgactctgacgtgtgtggaggacaccctgaaccccccgctttcaaacaagttttcaaattgtttgaggtcaggatttctcaaactgattcctttctttgcatatgagtatttgaaaataaatattttcccagaatataaataaatcatcacatgattattttaactat

SEQ ID NO: 23 - RNA, 1407 nt, synthetic construct
  source 1..1407: mol_type = other RNA
agatcactaacaccatataacgctatcttcctccttctccgacattccagtactcattccacaagccaccatggaagaacctcagtccgatccgagcgtcgagcctcccctgtcacaggaaactttcagtgacctgtggaaactgctgcccgagaataatgtactttcgcctctgcctagccaagcaatggatgatctgatgctgtctccagatgacatcgaacagtggtttacagaggatccagggcccgatgaggcaccacgaatgccagaggcggccccacctgttgcacccgcacctgcggctccaacacccgcagcccccgcccccgctccaagctggcctctcagtagttccgtgccatcacagaagacctatcaaggcagctacggatttcgcctcggatttctccattcaggcactgccaagtccgtgacttgtacgtacagccccgctctgaacaaaatgttctgtcagttggcgaagacatgtcctgtccagctttgggtagattctacccccccgccggggacacgggtgcgagccatggccatttataaacagtctcagcacatgaccgaggtcgtgcgcaggtgtcctcaccatgaacgatgctccgactccgacggcctggcccccccacagcacctgattcgcgtggaaggcaatcttcgtgtggagtacctcgatgatcggaacaccttcagacatagcgtggttgtgccttatgagccacccgaagttggaagcgactgtaccaccatccattacaactatatgtgcaacagtagctgcatgggtggcatgaatcggcggcctatcttgacaataatcactttagaggactcttccggaaacctgcttggcagaaattcattcgaggtccgtgtctgcgcctgcccgggcagggaccgcagaaccgaagaggagaatttacggaaaaagggggaaccccaccacgaactgccaccgggcagtaccaaaagggctctccctaataacacatcttcatcgccccagccaaagaagaaacccctcgacggagagtactttactctacaaattagggggagagaaagatttgagatgttccgcgaattgaacgaggccctggagttgaaagacgctcaagccggaaaggaaccaggtgggtctagggcccactcaagccatctgaagagtaagaaaggccagtccacttccaggcacaaaaagttaatgttcaagacggagggtcctgactctgacgtgtgtggaggacaccctgaaccccccgctttcaaacaagttttcaaattgtttgaggtcaggatttctcaaactgattcctttctttgcatatgagtatttgaaaataaatattttcccagaatataaataaatcatcacatgattattttaactat

SEQ ID NO: 24 - RNA, 1407 nt, synthetic construct
  source 1..1407: mol_type = other RNA
agtacccactccagataaactgacaaccatacgcgaacaacgacgaatcgtatcacacgcagaagccaccatggaagaacctcagtccgatccgagcgtcgagcctcccctgtcacaggaaactttcagtgacctgtggaaactgctgcccgagaataatgtactttcgcctctgcctagccaagcaatggatgatctgatgctgtctccagatgacatcgaacagtggtttacagaggatccagggcccgatgaggcaccacgaatgccagaggcggccccacctgttgcacccgcacctgcggctccaacacccgcagcccccgcccccgctccaagctggcctctcagtagttccgtgccatcacagaagacctatcaaggcagctacggatttcgcctcggatttctccattcaggcactgccaagtccgtgacttgtacgtacagccccgctctgaacaaaatgttctgtcagttggcgaagacatgtcctgtccagctttgggtagattctacccccccgccggggacacgggtgcgagccatggccatttataaacagtctcagcacatgaccgaggtcgtgcgcaggtgtcctcaccatgaacgatgctccgactccgacggcctggcccccccacagcacctgattcgcgtggaaggcaatcttcgtgtggagtacctcgatgatcggaacaccttcagacatagcgtggttgtgccttatgagccacccgaagttggaagcgactgtaccaccatccattacaactatatgtgcaacagtagctgcatgggtggcatgaatcggcggcctatcttgacaataatcactttagaggactcttccggaaacctgcttggcagaaattcattcgaggtccgtgtctgcgcctgcccgggcagggaccgcagaaccgaagaggagaatttacggaaaaagggggaaccccaccacgaactgccaccgggcagtaccaaaagggctctccctaataacacatcttcatcgccccagccaaagaagaaacccctcgacggagagtactttactctacaaattagggggagagaaagatttgagatgttccgcgaattgaacgaggccctggagttgaaagacgctcaagccggaaaggaaccaggtgggtctagggcccactcaagccatctgaagagtaagaaaggccagtccacttccaggcacaaaaagttaatgttcaagacggagggtcctgactctgacgtgtgtggaggacaccctgaaccccccgctttcaaacaagttttcaaattgtttgaggtcaggatttctcaaactgattcctttctttgcatatgagtatttgaaaataaatattttcccagaatataaataaatcatcacatgattattttaactat

SEQ ID NO: 25 - RNA, 1407 nt, synthetic construct
  source 1..1407: mol_type = other RNA
agcgagataacttacaaggagagagaagacgaggagagataaattagagagaaaacgagtaagagccaccatggaagaacctcagtccgatccgagcgtcgagcctcccctgtcacaggaaactttcagtgacctgtggaaactgctgcccgagaataatgtactttcgcctctgcctagccaagcaatggatgatctgatgctgtctccagatgacatcgaacagtggtttacagaggatccagggcccgatgaggcaccacgaatgccagaggcggccccacctgttgcacccgcacctgcggctccaacacccgcagcccccgcccccgctccaagctggcctctcagtagttccgtgccatcacagaagacctatcaaggcagctacggatttcgcctcggatttctccattcaggcactgccaagtccgtgacttgtacgtacagccccgctctgaacaaaatgttctgtcagttggcgaagacatgtcctgtccagctttgggtagattctacccccccgccggggacacgggtgcgagccatggccatttataaacagtctcagcacatgaccgaggtcgtgcgcaggtgtcctcaccatgaacgatgctccgactccgacggcctggcccccccacagcacctgattcgcgtggaaggcaatcttcgtgtggagtacctcgatgatcggaacaccttcagacatagcgtggttgtgccttatgagccacccgaagttggaagcgactgtaccaccatccattacaactatatgtgcaacagtagctgcatgggtggcatgaatcggcggcctatcttgacaataatcactttagaggactcttccggaaacctgcttggcagaaattcattcgaggtccgtgtctgcgcctgcccgggcagggaccgcagaaccgaagaggagaatttacggaaaaagggggaaccccaccacgaactgccaccgggcagtaccaaaagggctctccctaataacacatcttcatcgccccagccaaagaagaaacccctcgacggagagtactttactctacaaattagggggagagaaagatttgagatgttccgcgaattgaacgaggccctggagttgaaagacgctcaagccggaaaggaaccaggtgggtctagggcccactcaagccatctgaagagtaagaaaggccagtccacttccaggcacaaaaagttaatgttcaagacggagggtcctgactctgacgtgtgtggaggacaccctgaaccccccgctttcaaacaagttttcaaattgtttgaggtcaggatttctcaaactgattcctttctttgcatatgagtatttgaaaataaatattttcccagaatataaataaatcatcacatgattattttaactat

SEQ ID NO: 26 - RNA, 1407 nt, synthetic construct
  source 1..1407: mol_type = other RNA
agtaaactaaccactccatcacgtatatattcctctttcacacctttccattctcgaactaaccgccaccatggaagaacctcagtccgatccgagcgtcgagcctcccctgtcacaggaaactttcagtgacctgtggaaactgctgcccgagaataatgtactttcgcctctgcctagccaagcaatggatgatctgatgctgtctccagatgacatcgaacagtggtttacagaggatccagggcccgatgaggcaccacgaatgccagaggcggccccacctgttgcacccgcacctgcggctccaacacccgcagcccccgcccccgctccaagctggcctctcagtagttccgtgccatcacagaagacctatcaaggcagctacggatttcgcctcggatttctccattcaggcactgccaagtccgtgacttgtacgtacagccccgctctgaacaaaatgttctgtcagttggcgaagacatgtcctgtccagctttgggtagattctacccccccgccggggacacgggtgcgagccatggccatttataaacagtctcagcacatgaccgaggtcgtgcgcaggtgtcctcaccatgaacgatgctccgactccgacggcctggcccccccacagcacctgattcgcgtggaaggcaatcttcgtgtggagtacctcgatgatcggaacaccttcagacatagcgtggttgtgccttatgagccacccgaagttggaagcgactgtaccaccatccattacaactatatgtgcaacagtagctgcatgggtggcatgaatcggcggcctatcttgacaataatcactttagaggactcttccggaaacctgcttggcagaaattcattcgaggtccgtgtctgcgcctgcccgggcagggaccgcagaaccgaagaggagaatttacggaaaaagggggaaccccaccacgaactgccaccgggcagtaccaaaagggctctccctaataacacatcttcatcgccccagccaaagaagaaacccctcgacggagagtactttactctacaaattagggggagagaaagatttgagatgttccgcgaattgaacgaggccctggagttgaaagacgctcaagccggaaaggaaccaggtgggtctagggcccactcaagccatctgaagagtaagaaaggccagtccacttccaggcacaaaaagttaatgttcaagacggagggtcctgactctgacgtgtgtggaggacaccctgaaccccccgctttcaaacaagttttcaaattgtttgaggtcaggatttctcaaactgattcctttctttgcatatgagtatttgaaaataaatattttcccagaatataaataaatcatcacatgattattttaactat

SEQ ID NO: 27 - RNA, 1498 nt, synthetic construct
  source 1..1498: mol_type = other RNA
agtcctccccatcctctccctctgtccctctgtccctctgaccctgcactgtcccagcaccatggaagaacctcagtccgatccgagcgtcgagcctcccctgtcacaggaaactttcagtgacctgtggaaactgctgcccgagaataatgtactttcgcctctgcctagccaagcaatggatgatctgatgctgtctccagatgacatcgaacagtggtttacagaggatccagggcccgatgaggcaccacgaatgccagaggcggccccacctgttgcacccgcacctgcggctccaacacccgcagcccccgcccccgctccaagctggcctctcagtagttccgtgccatcacagaagacctatcaaggcagctacggatttcgcctcggatttctccattcaggcactgccaagtccgtgacttgtacgtacagccccgctctgaacaaaatgttctgtcagttggcgaagacatgtcctgtccagctttgggtagattctacccccccgccggggacacgggtgcgagccatggccatttataaacagtctcagcacatgaccgaggtcgtgcgcaggtgtcctcaccatgaacgatgctccgactccgacggcctggcccccccacagcacctgattcgcgtggaaggcaatcttcgtgtggagtacctcgatgatcggaacaccttcagacatagcgtggttgtgccttatgagccacccgaagttggaagcgactgtaccaccatccattacaactatatgtgcaacagtagctgcatgggtggcatgaatcggcggcctatcttgacaataatcactttagaggactcttccggaaacctgcttggcagaaattcattcgaggtccgtgtctgcgcctgcccgggcagggaccgcagaaccgaagaggagaatttacggaaaaagggggaaccccaccacgaactgccaccgggcagtaccaaaagggctctccctaataacacatcttcatcgccccagccaaagaagaaacccctcgacggagagtactttactctacaaattagggggagagaaagatttgagatgttccgcgaattgaacgaggccctggagttgaaagacgctcaagccggaaaggaaccaggtgggtctagggcccactcaagccatctgaagagtaagaaaggccagtccacttccaggcacaaaaagttaatgttcaagacggagggtcctgactctgacgtgtgtggaggacaccctgaaccccccgctttcaaacaagttttcaaattgtttgaggtcaggatttctcaaactgattcctttctttgcatatgagtatttgaaaataaatattttcccagaatataaataaatcatcacatgattattttaactataaaaaaaaaaaaaaaaaaaaaaaaaaaaaaaaaaaaaaaaaaaaaaaaaaaaaaaaaaaaaaaaaaaaaaaaaaaaaaaaaaaaaaaaaaaaaaaaaaaa

SEQ ID NO: 28 - RNA, 1487 nt, synthetic construct
  source 1..1487: mol_type = other RNA
agccgtcttccatcgttacagtcaccgttttcgcattctgtctagccaccatggaagaacctcagtccgatccgagcgtcgagcctcccctgtcacaggaaactttcagtgacctgtggaaactgctgcccgagaataatgtactttcgcctctgcctagccaagcaatggatgatctgatgctgtctccagatgacatcgaacagtggtttacagaggatccagggcccgatgaggcaccacgaatgccagaggcggccccacctgttgcacccgcacctgcggctccaacacccgcagcccccgcccccgctccaagctggcctctcagtagttccgtgccatcacagaagacctatcaaggcagctacggatttcgcctcggatttctccattcaggcactgccaagtccgtgacttgtacgtacagccccgctctgaacaaaatgttctgtcagttggcgaagacatgtcctgtccagctttgggtagattctacccccccgccggggacacgggtgcgagccatggccatttataaacagtctcagcacatgaccgaggtcgtgcgcaggtgtcctcaccatgaacgatgctccgactccgacggcctggcccccccacagcacctgattcgcgtggaaggcaatcttcgtgtggagtacctcgatgatcggaacaccttcagacatagcgtggttgtgccttatgagccacccgaagttggaagcgactgtaccaccatccattacaactatatgtgcaacagtagctgcatgggtggcatgaatcggcggcctatcttgacaataatcactttagaggactcttccggaaacctgcttggcagaaattcattcgaggtccgtgtctgcgcctgcccgggcagggaccgcagaaccgaagaggagaatttacggaaaaagggggaaccccaccacgaactgccaccgggcagtaccaaaagggctctccctaataacacatcttcatcgccccagccaaagaagaaacccctcgacggagagtactttactctacaaattagggggagagaaagatttgagatgttccgcgaattgaacgaggccctggagttgaaagacgctcaagccggaaaggaaccaggtgggtctagggcccactcaagccatctgaagagtaagaaaggccagtccacttccaggcacaaaaagttaatgttcaagacggagggtcctgactctgacgtgtgtggaggacaccctgaaccccccgctttcaaacaagttttcaaattgtttgaggtcaggatttctcaaactgattcctttctttgcatatgagtatttgaaaataaatattttcccagaatataaataaatcatcacatgattattttaactataaaaaaaaaaaaaaaaaaaaaaaaaaaaaaaaaaaaaaaaaaaaaaaaaaaaaaaaaaaaaaaaaaaaaaaaaaaaaaaaaaaaaaaaaaaaaaaaaaaa

SEQ ID NO: 29 - RNA, 1487 nt, synthetic construct
  source 1..1487: mol_type = other RNA
agaatccagtcaacgcatatccacgtatacccgaacacatcacagccaccatggaagaacctcagtccgatccgagcgtcgagcctcccctgtcacaggaaactttcagtgacctgtggaaactgctgcccgagaataatgtactttcgcctctgcctagccaagcaatggatgatctgatgctgtctccagatgacatcgaacagtggtttacagaggatccagggcccgatgaggcaccacgaatgccagaggcggccccacctgttgcacccgcacctgcggctccaacacccgcagcccccgcccccgctccaagctggcctctcagtagttccgtgccatcacagaagacctatcaaggcagctacggatttcgcctcggatttctccattcaggcactgccaagtccgtgacttgtacgtacagccccgctctgaacaaaatgttctgtcagttggcgaagacatgtcctgtccagctttgggtagattctacccccccgccggggacacgggtgcgagccatggccatttataaacagtctcagcacatgaccgaggtcgtgcgcaggtgtcctcaccatgaacgatgctccgactccgacggcctggcccccccacagcacctgattcgcgtggaaggcaatcttcgtgtggagtacctcgatgatcggaacaccttcagacatagcgtggttgtgccttatgagccacccgaagttggaagcgactgtaccaccatccattacaactatatgtgcaacagtagctgcatgggtggcatgaatcggcggcctatcttgacaataatcactttagaggactcttccggaaacctgcttggcagaaattcattcgaggtccgtgtctgcgcctgcccgggcagggaccgcagaaccgaagaggagaatttacggaaaaagggggaaccccaccacgaactgccaccgggcagtaccaaaagggctctccctaataacacatcttcatcgccccagccaaagaagaaacccctcgacggagagtactttactctacaaattagggggagagaaagatttgagatgttccgcgaattgaacgaggccctggagttgaaagacgctcaagccggaaaggaaccaggtgggtctagggcccactcaagccatctgaagagtaagaaaggccagtccacttccaggcacaaaaagttaatgttcaagacggagggtcctgactctgacgtgtgtggaggacaccctgaaccccccgctttcaaacaagttttcaaattgtttgaggtcaggatttctcaaactgattcctttctttgcatatgagtatttgaaaataaatattttcccagaatataaataaatcatcacatgattattttaactataaaaaaaaaaaaaaaaaaaaaaaaaaaaaaaaaaaaaaaaaaaaaaaaaaaaaaaaaaaaaaaaaaaaaaaaaaaaaaaaaaaaaaaaaaaaaaaaaaaa

SEQ ID NO: 30 - RNA, 1487 nt, synthetic construct
  source 1..1487: mol_type = other RNA
agccccccaacactgacttaatcgctttaagttcctccaaacgagccaccatggaagaacctcagtccgatccgagcgtcgagcctcccctgtcacaggaaactttcagtgacctgtggaaactgctgcccgagaataatgtactttcgcctctgcctagccaagcaatggatgatctgatgctgtctccagatgacatcgaacagtggtttacagaggatccagggcccgatgaggcaccacgaatgccagaggcggccccacctgttgcacccgcacctgcggctccaacacccgcagcccccgcccccgctccaagctggcctctcagtagttccgtgccatcacagaagacctatcaaggcagctacggatttcgcctcggatttctccattcaggcactgccaagtccgtgacttgtacgtacagccccgctctgaacaaaatgttctgtcagttggcgaagacatgtcctgtccagctttgggtagattctacccccccgccggggacacgggtgcgagccatggccatttataaacagtctcagcacatgaccgaggtcgtgcgcaggtgtcctcaccatgaacgatgctccgactccgacggcctggcccccccacagcacctgattcgcgtggaaggcaatcttcgtgtggagtacctcgatgatcggaacaccttcagacatagcgtggttgtgccttatgagccacccgaagttggaagcgactgtaccaccatccattacaactatatgtgcaacagtagctgcatgggtggcatgaatcggcggcctatcttgacaataatcactttagaggactcttccggaaacctgcttggcagaaattcattcgaggtccgtgtctgcgcctgcccgggcagggaccgcagaaccgaagaggagaatttacggaaaaagggggaaccccaccacgaactgccaccgggcagtaccaaaagggctctccctaataacacatcttcatcgccccagccaaagaagaaacccctcgacggagagtactttactctacaaattagggggagagaaagatttgagatgttccgcgaattgaacgaggccctggagttgaaagacgctcaagccggaaaggaaccaggtgggtctagggcccactcaagccatctgaagagtaagaaaggccagtccacttccaggcacaaaaagttaatgttcaagacggagggtcctgactctgacgtgtgtggaggacaccctgaaccccccgctttcaaacaagttttcaaattgtttgaggtcaggatttctcaaactgattcctttctttgcatatgagtatttgaaaataaatattttcccagaatataaataaatcatcacatgattattttaactataaaaaaaaaaaaaaaaaaaaaaaaaaaaaaaaaaaaaaaaaaaaaaaaaaaaaaaaaaaaaaaaaaaaaaaaaaaaaaaaaaaaaaaaaaaaaaaaaaaa

SEQ ID NO: 31 - RNA, 1487 nt, synthetic construct
  source 1..1487: mol_type = other RNA
agagcagaacgcgtaaccacaccatcgcaacatcccacttgatagccaccatggaagaacctcagtccgatccgagcgtcgagcctcccctgtcacaggaaactttcagtgacctgtggaaactgctgcccgagaataatgtactttcgcctctgcctagccaagcaatggatgatctgatgctgtctccagatgacatcgaacagtggtttacagaggatccagggcccgatgaggcaccacgaatgccagaggcggccccacctgttgcacccgcacctgcggctccaacacccgcagcccccgcccccgctccaagctggcctctcagtagttccgtgccatcacagaagacctatcaaggcagctacggatttcgcctcggatttctccattcaggcactgccaagtccgtgacttgtacgtacagccccgctctgaacaaaatgttctgtcagttggcgaagacatgtcctgtccagctttgggtagattctacccccccgccggggacacgggtgcgagccatggccatttataaacagtctcagcacatgaccgaggtcgtgcgcaggtgtcctcaccatgaacgatgctccgactccgacggcctggcccccccacagcacctgattcgcgtggaaggcaatcttcgtgtggagtacctcgatgatcggaacaccttcagacatagcgtggttgtgccttatgagccacccgaagttggaagcgactgtaccaccatccattacaactatatgtgcaacagtagctgcatgggtggcatgaatcggcggcctatcttgacaataatcactttagaggactcttccggaaacctgcttggcagaaattcattcgaggtccgtgtctgcgcctgcccgggcagggaccgcagaaccgaagaggagaatttacggaaaaagggggaaccccaccacgaactgccaccgggcagtaccaaaagggctctccctaataacacatcttcatcgccccagccaaagaagaaacccctcgacggagagtactttactctacaaattagggggagagaaagatttgagatgttccgcgaattgaacgaggccctggagttgaaagacgctcaagccggaaaggaaccaggtgggtctagggcccactcaagccatctgaagagtaagaaaggccagtccacttccaggcacaaaaagttaatgttcaagacggagggtcctgactctgacgtgtgtggaggacaccctgaaccccccgctttcaaacaagttttcaaattgtttgaggtcaggatttctcaaactgattcctttctttgcatatgagtatttgaaaataaatattttcccagaatataaataaatcatcacatgattattttaactataaaaaaaaaaaaaaaaaaaaaaaaaaaaaaaaaaaaaaaaaaaaaaaaaaaaaaaaaaaaaaaaaaaaaaaaaaaaaaaaaaaaaaaaaaaaaaaaaaaa

SEQ ID NO: 32 - RNA, 1507 nt, synthetic construct
  source 1..1507: mol_type = other RNA
agaccagacacctaacagactagacattttaccgaaatccgcattaaccattctaactcgtatagccaccatggaagaacctcagtccgatccgagcgtcgagcctcccctgtcacaggaaactttcagtgacctgtggaaactgctgcccgagaataatgtactttcgcctctgcctagccaagcaatggatgatctgatgctgtctccagatgacatcgaacagtggtttacagaggatccagggcccgatgaggcaccacgaatgccagaggcggccccacctgttgcacccgcacctgcggctccaacacccgcagcccccgcccccgctccaagctggcctctcagtagttccgtgccatcacagaagacctatcaaggcagctacggatttcgcctcggatttctccattcaggcactgccaagtccgtgacttgtacgtacagccccgctctgaacaaaatgttctgtcagttggcgaagacatgtcctgtccagctttgggtagattctacccccccgccggggacacgggtgcgagccatggccatttataaacagtctcagcacatgaccgaggtcgtgcgcaggtgtcctcaccatgaacgatgctccgactccgacggcctggcccccccacagcacctgattcgcgtggaaggcaatcttcgtgtggagtacctcgatgatcggaacaccttcagacatagcgtggttgtgccttatgagccacccgaagttggaagcgactgtaccaccatccattacaactatatgtgcaacagtagctgcatgggtggcatgaatcggcggcctatcttgacaataatcactttagaggactcttccggaaacctgcttggcagaaattcattcgaggtccgtgtctgcgcctgcccgggcagggaccgcagaaccgaagaggagaatttacggaaaaagggggaaccccaccacgaactgccaccgggcagtaccaaaagggctctccctaataacacatcttcatcgccccagccaaagaagaaacccctcgacggagagtactttactctacaaattagggggagagaaagatttgagatgttccgcgaattgaacgaggccctggagttgaaagacgctcaagccggaaaggaaccaggtgggtctagggcccactcaagccatctgaagagtaagaaaggccagtccacttccaggcacaaaaagttaatgttcaagacggagggtcctgactctgacgtgtgtggaggacaccctgaaccccccgctttcaaacaagttttcaaattgtttgaggtcaggatttctcaaactgattcctttctttgcatatgagtatttgaaaataaatattttcccagaatataaataaatcatcacatgattattttaactataaaaaaaaaaaaaaaaaaaaaaaaaaaaaaaaaaaaaaaaaaaaaaaaaaaaaaaaaaaaaaaaaaaaaaaaaaaaaaaaaaaaaaaaaaaaaaaaaaaa

SEQ ID NO: 33 - RNA, 1507 nt, synthetic construct
  source 1..1507: mol_type = other RNA
agatcactaacaccatataacgctatcttcctccttctccgacattccagtactcattccacaagccaccatggaagaacctcagtccgatccgagcgtcgagcctcccctgtcacaggaaactttcagtgacctgtggaaactgctgcccgagaataatgtactttcgcctctgcctagccaagcaatggatgatctgatgctgtctccagatgacatcgaacagtggtttacagaggatccagggcccgatgaggcaccacgaatgccagaggcggccccacctgttgcacccgcacctgcggctccaacacccgcagcccccgcccccgctccaagctggcctctcagtagttccgtgccatcacagaagacctatcaaggcagctacggatttcgcctcggatttctccattcaggcactgccaagtccgtgacttgtacgtacagccccgctctgaacaaaatgttctgtcagttggcgaagacatgtcctgtccagctttgggtagattctacccccccgccggggacacgggtgcgagccatggccatttataaacagtctcagcacatgaccgaggtcgtgcgcaggtgtcctcaccatgaacgatgctccgactccgacggcctggcccccccacagcacctgattcgcgtggaaggcaatcttcgtgtggagtacctcgatgatcggaacaccttcagacatagcgtggttgtgccttatgagccacccgaagttggaagcgactgtaccaccatccattacaactatatgtgcaacagtagctgcatgggtggcatgaatcggcggcctatcttgacaataatcactttagaggactcttccggaaacctgcttggcagaaattcattcgaggtccgtgtctgcgcctgcccgggcagggaccgcagaaccgaagaggagaatttacggaaaaagggggaaccccaccacgaactgccaccgggcagtaccaaaagggctctccctaataacacatcttcatcgccccagccaaagaagaaacccctcgacggagagtactttactctacaaattagggggagagaaagatttgagatgttccgcgaattgaacgaggccctggagttgaaagacgctcaagccggaaaggaaccaggtgggtctagggcccactcaagccatctgaagagtaagaaaggccagtccacttccaggcacaaaaagttaatgttcaagacggagggtcctgactctgacgtgtgtggaggacaccctgaaccccccgctttcaaacaagttttcaaattgtttgaggtcaggatttctcaaactgattcctttctttgcatatgagtatttgaaaataaatattttcccagaatataaataaatcatcacatgattattttaactataaaaaaaaaaaaaaaaaaaaaaaaaaaaaaaaaaaaaaaaaaaaaaaaaaaaaaaaaaaaaaaaaaaaaaaaaaaaaaaaaaaaaaaaaaaaaaaaaaaa

SEQ ID NO: 34 - RNA, 1507 nt, synthetic construct
  source 1..1507: mol_type = other RNA
agtacccactccagataaactgacaaccatacgcgaacaacgacgaatcgtatcacacgcagaagccaccatggaagaacctcagtccgatccgagcgtcgagcctcccctgtcacaggaaactttcagtgacctgtggaaactgctgcccgagaataatgtactttcgcctctgcctagccaagcaatggatgatctgatgctgtctccagatgacatcgaacagtggtttacagaggatccagggcccgatgaggcaccacgaatgccagaggcggccccacctgttgcacccgcacctgcggctccaacacccgcagcccccgcccccgctccaagctggcctctcagtagttccgtgccatcacagaagacctatcaaggcagctacggatttcgcctcggatttctccattcaggcactgccaagtccgtgacttgtacgtacagccccgctctgaacaaaatgttctgtcagttggcgaagacatgtcctgtccagctttgggtagattctacccccccgccggggacacgggtgcgagccatggccatttataaacagtctcagcacatgaccgaggtcgtgcgcaggtgtcctcaccatgaacgatgctccgactccgacggcctggcccccccacagcacctgattcgcgtggaaggcaatcttcgtgtggagtacctcgatgatcggaacaccttcagacatagcgtggttgtgccttatgagccacccgaagttggaagcgactgtaccaccatccattacaactatatgtgcaacagtagctgcatgggtggcatgaatcggcggcctatcttgacaataatcactttagaggactcttccggaaacctgcttggcagaaattcattcgaggtccgtgtctgcgcctgcccgggcagggaccgcagaaccgaagaggagaatttacggaaaaagggggaaccccaccacgaactgccaccgggcagtaccaaaagggctctccctaataacacatcttcatcgccccagccaaagaagaaacccctcgacggagagtactttactctacaaattagggggagagaaagatttgagatgttccgcgaattgaacgaggccctggagttgaaagacgctcaagccggaaaggaaccaggtgggtctagggcccactcaagccatctgaagagtaagaaaggccagtccacttccaggcacaaaaagttaatgttcaagacggagggtcctgactctgacgtgtgtggaggacaccctgaaccccccgctttcaaacaagttttcaaattgtttgaggtcaggatttctcaaactgattcctttctttgcatatgagtatttgaaaataaatattttcccagaatataaataaatcatcacatgattattttaactataaaaaaaaaaaaaaaaaaaaaaaaaaaaaaaaaaaaaaaaaaaaaaaaaaaaaaaaaaaaaaaaaaaaaaaaaaaaaaaaaaaaaaaaaaaaaaaaaaaa

SEQ ID NO: 35 - RNA, 1507 nt, synthetic construct
  source 1..1507: mol_type = other RNA
agcgagataacttacaaggagagagaagacgaggagagataaattagagagaaaacgagtaagagccaccatggaagaacctcagtccgatccgagcgtcgagcctcccctgtcacaggaaactttcagtgacctgtggaaactgctgcccgagaataatgtactttcgcctctgcctagccaagcaatggatgatctgatgctgtctccagatgacatcgaacagtggtttacagaggatccagggcccgatgaggcaccacgaatgccagaggcggccccacctgttgcacccgcacctgcggctccaacacccgcagcccccgcccccgctccaagctggcctctcagtagttccgtgccatcacagaagacctatcaaggcagctacggatttcgcctcggatttctccattcaggcactgccaagtccgtgacttgtacgtacagccccgctctgaacaaaatgttctgtcagttggcgaagacatgtcctgtccagctttgggtagattctacccccccgccggggacacgggtgcgagccatggccatttataaacagtctcagcacatgaccgaggtcgtgcgcaggtgtcctcaccatgaacgatgctccgactccgacggcctggcccccccacagcacctgattcgcgtggaaggcaatcttcgtgtggagtacctcgatgatcggaacaccttcagacatagcgtggttgtgccttatgagccacccgaagttggaagcgactgtaccaccatccattacaactatatgtgcaacagtagctgcatgggtggcatgaatcggcggcctatcttgacaataatcactttagaggactcttccggaaacctgcttggcagaaattcattcgaggtccgtgtctgcgcctgcccgggcagggaccgcagaaccgaagaggagaatttacggaaaaagggggaaccccaccacgaactgccaccgggcagtaccaaaagggctctccctaataacacatcttcatcgccccagccaaagaagaaacccctcgacggagagtactttactctacaaattagggggagagaaagatttgagatgttccgcgaattgaacgaggccctggagttgaaagacgctcaagccggaaaggaaccaggtgggtctagggcccactcaagccatctgaagagtaagaaaggccagtccacttccaggcacaaaaagttaatgttcaagacggagggtcctgactctgacgtgtgtggaggacaccctgaaccccccgctttcaaacaagttttcaaattgtttgaggtcaggatttctcaaactgattcctttctttgcatatgagtatttgaaaataaatattttcccagaatataaataaatcatcacatgattattttaactataaaaaaaaaaaaaaaaaaaaaaaaaaaaaaaaaaaaaaaaaaaaaaaaaaaaaaaaaaaaaaaaaaaaaaaaaaaaaaaaaaaaaaaaaaaaaaaaaaaa

SEQ ID NO: 36 - RNA, 1507 nt, synthetic construct
  source 1..1507: mol_type = other RNA
agtaaactaaccactccatcacgtatatattcctctttcacacctttccattctcgaactaaccgccaccatggaagaacctcagtccgatccgagcgtcgagcctcccctgtcacaggaaactttcagtgacctgtggaaactgctgcccgagaataatgtactttcgcctctgcctagccaagcaatggatgatctgatgctgtctccagatgacatcgaacagtggtttacagaggatccagggcccgatgaggcaccacgaatgccagaggcggccccacctgttgcacccgcacctgcggctccaacacccgcagcccccgcccccgctccaagctggcctctcagtagttccgtgccatcacagaagacctatcaaggcagctacggatttcgcctcggatttctccattcaggcactgccaagtccgtgacttgtacgtacagccccgctctgaacaaaatgttctgtcagttggcgaagacatgtcctgtccagctttgggtagattctacccccccgccggggacacgggtgcgagccatggccatttataaacagtctcagcacatgaccgaggtcgtgcgcaggtgtcctcaccatgaacgatgctccgactccgacggcctggcccccccacagcacctgattcgcgtggaaggcaatcttcgtgtggagtacctcgatgatcggaacaccttcagacatagcgtggttgtgccttatgagccacccgaagttggaagcgactgtaccaccatccattacaactatatgtgcaacagtagctgcatgggtggcatgaatcggcggcctatcttgacaataatcactttagaggactcttccggaaacctgcttggcagaaattcattcgaggtccgtgtctgcgcctgcccgggcagggaccgcagaaccgaagaggagaatttacggaaaaagggggaaccccaccacgaactgccaccgggcagtaccaaaagggctctccctaataacacatcttcatcgccccagccaaagaagaaacccctcgacggagagtactttactctacaaattagggggagagaaagatttgagatgttccgcgaattgaacgaggccctggagttgaaagacgctcaagccggaaaggaaccaggtgggtctagggcccactcaagccatctgaagagtaagaaaggccagtccacttccaggcacaaaaagttaatgttcaagacggagggtcctgactctgacgtgtgtggaggacaccctgaaccccccgctttcaaacaagttttcaaattgtttgaggtcaggatttctcaaactgattcctttctttgcatatgagtatttgaaaataaatattttcccagaatataaataaatcatcacatgattattttaactataaaaaaaaaaaaaaaaaaaaaaaaaaaaaaaaaaaaaaaaaaaaaaaaaaaaaaaaaaaaaaaaaaaaaaaaaaaaaaaaaaaaaaaaaaaaaaaaaaaa